European Patent Application EP 4 628 087 A1, published October 8, 2025. Title: 局所投与用の医薬組成物. Applicant: 国立感染症研究所長が代表する日本国. The sequence listing filed with the application follows.

SEQUENCE LISTING (14 sequences)

SEQ ID NO: 1 - DNA, 20 bp, synthetic construct
  source 1..20: mol_type = other DNA
aaattttggggaccaggaac

SEQ ID NO: 2 - DNA, 20 bp, synthetic construct
  source 1..20: mol_type = other DNA
tggcagctgtgtaggtcaac

SEQ ID NO: 3 - DNA, 20 bp, synthetic construct
  source 1..20: mol_type = other DNA
atgtcgcgcattggcatgga

SEQ ID NO: 4 - DNA, 29 bp, synthetic construct
  source 1..29: mol_type = other DNA
ccmaggtcgaaacgtaygttctctctatc

SEQ ID NO: 5 - DNA, 32 bp, synthetic construct
  source 1..32: mol_type = other DNA
tgacagratyggtcttgtctttagccaytcca

SEQ ID NO: 6 - DNA, 22 bp, synthetic construct
  source 1..22: mol_type = other DNA
atytcggctttgagggggcctg

SEQ ID NO: 7 - DNA, 21 bp, synthetic construct
  source 1..21: mol_type = other DNA
cccgtgagtgtcaactaccac

SEQ ID NO: 8 - DNA, 21 bp, synthetic construct
  source 1..21: mol_type = other DNA
gcccaagtattcacccctgtc

SEQ ID NO: 9 - DNA, 21 bp, synthetic construct
  source 1..21: mol_type = other DNA
ggtgtccgtgactaactccat

SEQ ID NO: 10 - DNA, 22 bp, synthetic construct
  source 1..22: mol_type = other DNA
ctgtaccactagcatcactgtg

SEQ ID NO: 11 - DNA, 21 bp, synthetic construct
  source 1..21: mol_type = other DNA
gaccataggggtcttgaccaa

SEQ ID NO: 12 - DNA, 23 bp, synthetic construct
  source 1..23: mol_type = other DNA
agacttgctctttctgaaaagcc

SEQ ID NO: 13 - DNA, 21 bp, synthetic construct
  source 1..21: mol_type = other DNA
aggtcggtgtgaacggatttg

SEQ ID NO: 14 - DNA, 19 bp, synthetic construct
  source 1..19: mol_type = other DNA
ggggtcgttgatggcaaca